European Patent Specification EP 3 145 294 B1, published July 23, 2025. Title: Melon plants with whitefly resistance. Applicant: Nunhems B.V. The sequence listing filed with the application follows.

SEQUENCE LISTING (68 sequences)

SEQ ID NO: 1 - DNA, 101 bp, Cucumis melo
  variation (51)..(51): SNP mME20364
taagggttggttacgcaagggtcgactttcaatctgtttgagaaaacaagcggttcttagctmttgacctttatgataggtgccttgagaagggccctcrt

SEQ ID NO: 2 - DNA, 85 bp, Cucumis melo
  variation (35)..(35): SNP mME17490
gcatttttacagcatagaaaaactatggtcgggcaaattagggatgcaattacaaagagaaatttgatagagatggaagatgatt

SEQ ID NO: 3 - DNA, 84 bp, Cucumis melo
  variation (34)..(34): SNP mME15248
gtttggtatctgttgggatccatgattctgcatccttacttgtactggaacttgggagtgtttggaagtaggcagttatttccc

SEQ ID NO: 4 - DNA, 101 bp, Cucumis melo
  variation (51)..(51): SNP mME17306
taatggtgaaaaacaagattgctgacgataaattggtaccgaattatcaacacgaaaccaaacaaaaacttggctaagttatgggattggataggcattcc

SEQ ID NO: 5 - DNA, 101 bp, Cucumis melo
  variation (51)..(51): SNP mME26059
acaaaaagtataacacatcaatatacgtggaaacttgtaaagggagaaaaactacgatrgagacttttcttattattttcttatgaaacatgaagatacaa

SEQ ID NO: 6 - DNA, 83 bp, Cucumis melo
  variation (33)..(33): SNP mME38084
gccgtgtagcgtctctctctaaaacagacattgccataaaatttcagaaaaagaaacaaattacgaacataaaaccaaagcat

SEQ ID NO: 7 - DNA, 99 bp, Cucumis melo
  variation (51)..(51): SNP mME21974
ttagcggcatgcaaattcactttatccaaaggattgattccgatggtcttcgaggccagatgcgacattggcggcgbttggacrgagacgctrsacggc

SEQ ID NO: 8 - DNA, 101 bp, Cucumis melo
  variation (51)..(51): SNP mME12777
tgcggcgaagaatcacacagtctgtaggagtacaataaggattcaaacaacttagaaggaaaatcaatagagcacgattctatgatactcctcaaaattga

SEQ ID NO: 9 - DNA, 101 bp, Cucumis melo
  variation (51)..(51): SNP mME15151
ttctttaacagttcttgattcgtgggtctctttcttttgttgaatgtagagcgttcttccttgtcattgtggtagaaagaaagtgaattgaaactttaaag

SEQ ID NO: 10 - DNA, 101 bp, Cucumis melo
  variation (51)..(51): SNP mME26139
atttaaatgctaataaatatcatatatacagaaacaaatgactatgacgtcaaattagagtagaaattacctgcttgatacaatataggacagaactgtaa

SEQ ID NO: 11 - DNA, 101 bp, Cucumis melo
  variation (51)..(51): SNP mME48762
tttcgaagcatcgtttacaagctgttcctgtggttgagctttccaattctcacgtaattggtttcattacacaggtacttactactggttttaacaacccc

SEQ ID NO: 12 - DNA, 101 bp, Cucumis melo
  variation (51)..(51): SNP mME25039
gagggaagatagttaaacaactcggataatgagagagaaaccacagaaaccatggttctttcattgcatacttaaactaratcaatttggaccttaggttt

SEQ ID NO: 13 - DNA, 101 bp, Cucumis melo
  variation (51)..(51): SNP mME40109
ttcattgcaagagtcaacagatagcggtgaagatggacaagctargaagcttaaaggtggctctaggcttacttctgatgcagccaatattgatatcattc

SEQ ID NO: 14 - DNA, 192 bp, Cucumis melo
catcttacaaaatgtatcagaggcatttctaaacttttttaaatgagcaaaagtcttgaaaagcagatcaaaaacatgcggcgaagaatcacacagtctgtaggagtacaataaggattcaaacaacttagaaggaaaatcaatagagcacgattctatgatactcctcaaaattgattctgcakgtacgca

SEQ ID NO: 15 - DNA, 1485 bp, Cucumis melo
ttttttttctcttctttaacagttcttgattcgtgggtctctttcttttgttgaatgtagaacgttcttccttgtcattgtggtagaaagaaagtgaattgaaactttaaagctagttgtttaattgctctgttctgccaaatgagaccttgtttcttgctttggaattgtttatgaatgccgaaactgwtatcgtaagaattggttttyaatgtcaagaatctatttggcatgtttcggttatgcttttcttgaattttctagaagttttcctcttatatgaattcttgtaaacaattttggctttgggagttataatgctgaaggatattctccctttgtctgtctcttcttgtcactctgctcaaaagcaatatgattatgaacttttacctttagttccatggctgtaatcgtaatgctttggtttgaattgaacttcaagtcatgatatattggattagctttgaaatatttgatggttgtatttgtggcatccagcatgtctcaatatggtaaagaaggttagagtcattgagtaacctttccattttttgtttttagttttgataaatatgtctatttggaaagtattcgttgtttgccatatcttgatgtttctaataactgtactccaatttggaaatcaaaacaaaatacttttcttgttttgttatgtcaatgtgtaacaatccaaagttagtatcaagagaatcataagcaacaaataaaaaatgaggaagatatgaaatgagcctaatttatcatcagtcgaagtactgaagttgtgtgtatttcttcagttgtatagatgggttgttgctagaaccacaaagcttttcttgtttcctttgcactctcagttgcctgagaaaacccgagaggatatcatagtactaaatgtaggttctataatatgacgataatcatttggtttatgttctgttacattactggttacatttaataaaactccaggacgatatagtatttgttggatatatttgcatacctagctatatattataagatgcagataattctttcagctataattgactttrtttctcttgtgattttaaggatttgcaacaacagcaacaatatgaacggggagctgccctcaatgagatcgaacacagccgcaagatcctacttgacaagctcaaggattacaaaggagagtatttggaagtggtaaaggaagcttctgccttcgctggggaggcagtaaagaacaaccatgacctcatgcttccyccatatccaagtcgctccmcatatcctcttcacctagacaatgaccatttatcaccattcgtrtctgctcgcaaatctgcccgtaatggggtaaccttgagctacatgacaaatgatgccaaaagagagtcaagcgagtcactaagtaccagcaaagaagcgagcacgaaaaacacaaggaatggattaggttcactcatagctgcakgtacgccgtctagactg

SEQ ID NO: 16 - DNA, 134 bp, Cucumis melo
gtttggtatctgttgggatccatgattctgcatccttacttgtactggaacttgggagtgtttggaagtaggcagttatttcccatttgcaatctgttataagaaggtaaaattataaaagttctttcaatttt

SEQ ID NO: 17 - DNA, 1871 bp, Cucumis melo
gctacacggctgcaacaagaaaatgagagggccaattacttagatttttcagttgttagttttgaacatttcgtttgcataaatcaaaaagtctcttacatgtctccacttatggccaagaaactcattcacagctattccattttgtgcatacatcattggagaggtccagtagccccaaatccaccaaggatgcacatcatctaaacataaagagaagttctcattttaagtaatttttcttatgtaatggtattgaaaacacataggtcacttgaatcaaacctcgagctaagacaaatccacccaaaacaagaactgtaagtaaagcaaatgatccaaatgtatttgcaacgatgatattccgtcccaatgctccaatcaaacggaacagcgcagatgccatttggttcacacacaggagcaggagaaaatgtttgaagaatctgcaagtccatcatacgacctaatgttatcaagaaggtaaaataatcaaattggtagttcagtgttagtgttcttcattttcttgtaccttccggcgtttggatcgaatccaacgacatagtaagtcattaccacccaaattccaacttcgacaaaagtaatagggatcttaaggatccatgtgggtatagaatatgcccaagggggaaagaagaggaagtccctttgcttgtagaacacaggaagtttcaagattgtcaaagcaagctcagagaaaccattgaacatgattatgataatcgcaaagaacaatgctcccatgtaaaccgatccatcatctactgtcctccggcgcatctcggttcggaaaaacaaggtcattgtcacaaaagccatcagaatgagctgaaaaatgaagaaacatagtagtgtcaaacatgagctatcggagagtgaataaagatatgaactacggaactaaaactcacttgagtcaacttgaaaatgtacacaaatgagtttctcttcatgagtaaaagctcccttgaaatgcaagctttcaacagttccttcttgctagcaccatacttctcggttgttaaagcagcagggtggcttttagayttgtcaaatggagtggcaagctcatcacctagcttcttccccacatgaaatgattgaaaggcttcagaaaactcctccacactgacaaatctataaacctcatctctcttagtccaatattgttcttgatctttccttgaagtgacctataaaacagtttccatcagccaaacaaaatggatgaaasaaatagcagaaaagaacacattatgaaaatggggaaagttaaaaggccaaacgagcttacttcttgtaagaagtcagctactcctttcctctgagggcaagtgaagcccatatgttggaagaactcgagcacgttttcacgtggaccttgatacacaacttgtccatctgatatcagaattatgtcatcaaacaattcataagtttcaggggmcggwtgaagaagagagatcagagcagttccattcagaatatgaatggactgtctcattgaattaacaatctgatacgttgtcgaactgtccaatcctgtcgatatctcgtccatgaacagagctctcgctggtccaaccaacatctccccagtcgtcaccctcttcttttgcccaccggagatccctcgaaacatttcatctcctaccattgtgtcagcacrgatttcaagtcctagaatctgcataaacaatcaaaaaaacattataagaccatatactattagtttmtttgctgcttagtttttttgctgcttagttattattacaaaaagttttcacctttagtacataatctgtcactacattggtttcttgtcctcctaaagctgcakgtacgca

SEQ ID NO: 18 - DNA, 201 bp, Cucumis melo
tcctaaggtaatctgagagacgttcaatttcagactgttcaaaggatccctaatggtgaaaaacaagattgctgacgataaattggtaccgaattatcaacacgaaaccaaacaaaaacttggctaagttatgggattggataggcattccgcttttgacttttctatcattggattgaactcgaaggaaatgcctcgatc

SEQ ID NO: 19 - DNA, 190 bp, Cucumis melo
gcatttttacagcatagaaaaactatggtcgggcaaattagggatgcaattacaaagagaaatttgatagagatggaagatgattagattacctggatgagagttagggctcctagtacaagaaaggtacataaaatgaatgacgccgtcttagccatttcgccskgtagcttctctatagagacgctac

SEQ ID NO: 20 - DNA, 1052 bp, Cucusmis melo
gcgtacmtgcagcggatgtactttgaagatccatatccattatcatcagatgatcgtaagggttggttacgcaagggtcgactttcaatctgtttgagaaaacaagcggttcttagctmttgacctttatgataggtgccttgagaagggccctcrtggtcattgggcaaaaataaatacctttgttaggttgatttggcgaagagcaaaaactgcaagtgccttgaagagaattcccggaccctcctctagtgagaaaactatacttgtctgaaaaggaagcgagcatattacatacaacaaygtacttattctaagcaccatatacatgaatgcaaagaattagaagggaagagactcttttcctcctaaaaawacgaaaggctaaccttgaatggcctatcaatgcctggaattatgggttctctcgctagcattagaaatcgagttacattgtcagagtcatcctaatagaagaaaagaaaattggtaatcggtgcagcattagaatgtatgggctagtaaatcataattaaatgcttaagtaaacacctgaatatcttcagcaagtatattcaagccatatatggacgcagccacsgagctagcaacagctcctgcatctttcaatttgtgaaaagcaacatgctgcacaatatcmaaagtctcatcaactatcattctgaaccagcaatcaaaatgatgaaaatttggatgatacgaatatataatcatcaatcatcaaaacttcatataagcattgctgataaataagcatcaacaaaaatctgatttgccttctcagaatcactatygagccattataataataaraaatgacaagttttcctgtagaatagaccaaaaaatgacaaaatatcataacagtaacggagcagcaattgaacagccaaagataaagtacctttgcagcaccagcagtatcgtccactgcttctctcaccaatcctagccctgtcaatgtgttttcacactgrgcmagagcctgaacaagaatcatgttaagccgkgtagcgtctcagactgcgtac

SEQ ID NO: 21 - DNA, 134 bp, Cucumis melo
ttcaaaagtagaaacaagagaattcaacttgtttcataaacatattccagattttccacaacaacaaataaacctaataatgaacacaatcgaattcaggcacagaacaaaggccacgatcggagttaaaaaaa

SEQ ID NO: 22 - DNA, 124 bp, Cucumis melo
agagacgctacmcggagtaagcggattagcggcatgcaaattcactttatccaaaggattgattccgatggtcttagaggccagatgcgacattggcggcgbttggacrgagacgctrsacggc

SEQ ID NO: 23 - DNA, 406 bp, Cucumis melo
aatttaaattttttgtcaaatatatacatcaatttacaccctgaacgtagatttcctagctaatcaatccagaccatttatcaaataatctatatctaattttactagatcccattcaaaatcaactcaaaattatctaaataaaattacttttcttcaaaaagtccccaagtagcagaaccaatagaaaacgggaaatttaatgaagtcgtaagttcaactttaacaatttttaaaacaaaattctaatagattgtttaaactgatttacttattaatttgagatttttgtggatacaagccgtaaaagttaaaaaaggggtataaatgaacttatattattcaaaatttatcaaatttattcataggaaatgaagcaccaaggaataccagaaaataawtgaca

SEQ ID NO: 24 - DNA, 585 bp, Cucumis melo
cgctacmcggttcagggccaagaatataagcccaaattgcattgtaatcaacagagctmctatttttaatcattgtggacycaacttgtgttaggtgtgtattaagcaatgccttgtcaagcacatttgaaatgacatgcaacccaaggacacgttgacctggtatctgacaccaacgagaagctagagtgaaaattattgaaagagacaaaaagtataacacatcaatatacgtggaaacttgtaaagggagaaaaactacgatrgagacttttcttattattttcttatgaaacatgaagatacaaaggcgaagaattaacaggcaacaaaagctttaacaaaaacggaaagaaacagtaggtaaaataatttacataaatacccttgagctttcaacatacaagaagcccataaattctgacagaaggtttaaagagttcaaaataacaaacttctagaagatttgaaataaatgaaaaaagagctatttcataacgaataagaaaaataaggggccaaaagtggaaaaaaacyaacagtattttatggttgaaaaaaattgtcactacaatgaagcaacta

SEQ ID NO: 25 - DNA, 133 bp, Cucumis melo
gccgtgtagcgtctctctctaaaacagacattaccataaaatttcagaaaaagaaacaaattacgaacataaaaccaaagcattaagagtagaatcaaataaatgaagaatccaatcacagaaacagcaggaa

SEQ ID NO: 26 - DNA, 201 bp, Cucumis melo
ttattttcctgttggaatgagggatacactttttcatgttcttcttatgttttcgaagcatcgtttacaagctgttcctgtggttgagctttccaattctaacgtaattggtttcattacacaggtacttactactggttttaacaaccccgtcgattacttttgactaatcttatgggacaacaccttttaacatttagg

SEQ ID NO: 27 - DNA, 49 bp, artificial
  primer mME12777
gaaggtgaccaagttcatgctgtaggagtacaataaggattcaaacaac

SEQ ID NO: 28 - DNA, 49 bp, artificial
  primer mME12777
gaaggtcggagtcaacggattgtaggagtacaataaggattcaaacaat

SEQ ID NO: 29 - DNA, 29 bp, artificial
  common primer mME12777
ggagtatcatagaatcgtgctctattgat

SEQ ID NO: 30 - DNA, 44 bp, artificial
  primer mME15151
gaaggtgaccaagttcatgctaccacaatgacaaggaagaacgt

SEQ ID NO: 31 - DNA, 44 bp, artificial
  primer mME15151
gaaggtcggagtcaacggattaccacaatgacaaggaagaacgc

SEQ ID NO: 32 - DNA, 29 bp, artificial
  common primer mME15151
tcgtgggtctctttcttttgttgaatgta

SEQ ID NO: 33 - DNA, 44 bp, artificial
  primer mME15248
gaaggtgaccaagttcatgctcccaagttccagtacaagtaagg

SEQ ID NO: 34 - DNA, 46 bp, artificial
  primer mME15248
gaaggtcggagtcaacggattctcccaagttccagtacaagtaaga

SEQ ID NO: 35 - DNA, 27 bp, artificial
  common primer mME15248
tatctgttgggatccatgattctgcat

SEQ ID NO: 36 - DNA, 43 bp, artificial
  primer mME17011
gaaggtgaccaagttcatgcttgtcgaactgtccaatcctgtc

SEQ ID NO: 37 - DNA, 45 bp, artificial
  primer mME17011
gaaggtcggagtcaacggattgttgtcgaactgtccaatcctgtt

SEQ ID NO: 38 - DNA, 25 bp, artificial
  common primer mME17011
gagagctctgttcatggacgagata

SEQ ID NO: 39 - DNA, 49 bp, artificial
  primer mME17306
gaaggtgaccaagttcatgctgacgataaattggtaccgaattatcaac

SEQ ID NO: 40 - DNA, 49 bp, artificial
  primer mME17306
gaaggtcggagtcaacggattgacgataaattggtaccgaattatcaat

SEQ ID NO: 41 - DNA, 29 bp, artificial
  common primer mME17306
ctatccaatcccataacttagccaagttt

SEQ ID NO: 42 - DNA, 46 bp, artificial
  primer mME17409
gaaggtgaccaagttcatgctagcatagaaaaactatggtcgggca

SEQ ID NO: 43 - DNA, 44 bp, artificial
  primer mME17490
gaaggtcggagtcaacggattcatagaaaaactatggtcgggcg

SEQ ID NO: 44 - DNA, 30 bp, artificial
  common primer mME17490
caaatttctctttgtaattgcatccctaat

SEQ ID NO: 45 - DNA, 49 bp, artificial
  primer mME20364
gaaggtgaccaagttcatgctgactttcaatctgtttgagaaaacaagc

SEQ ID NO: 46 - DNA, 50 bp, artificial
  primer mME20364
gaaggtcggagtcaacggattcgactttcaatctgtttgagaaaacaagt

SEQ ID NO: 47 - DNA, 27 bp, artificial
  common primer mME20364
ggcacctatcataaaggtcaakagcta

SEQ ID NO: 48 - DNA, 47 bp, artificial
  primer mME21134
gaaggtgaccaagttcatgctaataatgaacacaatcgaattcaggc

SEQ ID NO: 49 - DNA, 50 bp, artificial
  primer mME21134
gaaggtcggagtcaacggattcctaataatgaacacaatcgaattcaggt

SEQ ID NO: 50 - DNA, 28 bp, artificial
  common primer mME21134
ttttttaactccgatcgtggcctttgtt

SEQ ID NO: 51 - DNA, 42 bp, artificial
  primer mME21974
gaaggtgaccaagttcatgctccaatgtcgcatctggcctct

SEQ ID NO: 52 - DNA, 42 bp, artificial
  primer mME21974
gaaggtcggagtcaacggattccaatgtcgcatctggcctcg

SEQ ID NO: 53 - DNA, 29 bp, artificial
  common primer mME21974
ttatccaaaggattgattccgatggtctt

SEQ ID NO: 54 - DNA, 51 bp, artificial
  primer mME22724
gaaggtgaccaagttcatgctgtcaaatatatacatcaatttacaccctga

SEQ ID NO: 55 - DNA, 49 bp, artificial
  primer mME22724
gaaggtcggagtcaacggattcaaatatatacatcaatttacaccctgg

SEQ ID NO: 56 - DNA, 29 bp, artificial
  common primer mME22724
tggtctggattgattagctaggaaatcta

SEQ ID NO: 57 - DNA, 48 bp, artificial
  primer mME26059
gaaggtgaccaagttcatgctacgtggaaacttgtaaagggagaaaaa

SEQ ID NO: 58 - DNA, 48 bp, artificial
  primer mME26059
gaaggtcggagtcaacggattacgtggaaacttgtaaagggagaaaat

SEQ ID NO: 59 - DNA, 30 bp, artificial
  common primer mME26059
cgcctttgtatcttcatgtttcataagaaa

SEQ ID NO: 60 - DNA, 54 bp, artificial
  primer mME38084
gaaggtgaccaagttcatgctcgtaatttgtttctttttctgaaattttatggt

SEQ ID NO: 61 - DNA, 53 bp, artificial
  primer mME38084
gaaggtcggagtcaacggattgtaatttgtttctttttctgaaattttatggc

SEQ ID NO: 62 - DNA, 28 bp, artificial
  common primer mME38084
tgtagcgtctctctctaaaacagacatt

SEQ ID NO: 63 - DNA, 49 bp, artificial
  primer mME48762
gaaggtgaccaagttcatgctgtacctgtgtaatgaaaccaattacgtt

SEQ ID NO: 64 - DNA, 47 bp, artificial
  primer mME48762
gaaggtcggagtcaacggattacctgtgtaatgaaaccaattacgtg

SEQ ID NO: 65 - DNA, 25 bp, artificial
  common primer mME48762
ctgttcctgtggttgagctttccaa

SEQ ID NO: 66 - DNA, 101 bp, Cucumis melo
  variation (51)..(51): SNP mME17011
tgtctcattgaattaacaatctgatacgttgtcgaactgtccaatcctgttgatatctcgtccatgaacagagctctcgctggtccaaccaacatctcccc

SEQ ID NO: 67 - DNA, 94 bp, Cucumis melo
  variation (44)..(44): SNP mME22724
aatttaaattttttgtcaaatatatacatcaatttacaccctgaacgtagatttcctagctaatcaatccagaccatttatcaaataatctata

SEQ ID NO: 68 - DNA, 84 bp, Cucumis melo
  variation (51)..(51): SNP mME21134
attttccacaacaacaaataaacctaataatgaacacaatcgaattcaggtacagaacaaaggccacgatcggagttaaaaaaa